European Patent Specification EP 3 137 504 B1, published May 10, 2023. Title: ANTIBODY BINDING TO FCRN FOR TREATING AUTOIMMUNE DISEASES. Applicant: HANALL BIOPHARMA CO. LTD. The sequence listing filed with the application follows.

SEQUENCE LISTING (44 sequences)

SEQ ID NO: 1 - DNA, 363 bp, Artificial Sequence
  Hv of HL161A
gaagtgcagctgctggaatccggcggaggcctggtgcagcctggcggctctctgagactgtcctgcgccgcctccgagttcaccttcggcagctgcgtgatgacctgggtccgacaggctcccggcaagggcctggaatgggtgtccgtgatctccggctccggcggctccacctactacgccgactctgtgaagggccggttcaccatctcccgggacaactccaagaacaccctgtacctgcagatgaactccctgcgggccgaggacaccgccgtgtactactgcgccaagaccccctggtggctgcggtcccccttcttcgattactggggccagggcaccctggtgacagtgtcctcc

SEQ ID NO: 2 - protein, 121 aa, Artificial Sequence
  Hv of HL161A
EVQLLESGGGLVQPGGSLRLSCAASEFTFGSCVMTWVRQAPGKGLEWVSVISGSGGSTYYADSVKGRFTISRDNSKNTLYLQMNSLRAEDTAVYYCAKTPWWLRSPFFDYWGQGTLVTVSS

SEQ ID NO: 3 - DNA, 363 bp, Artificial Sequence
  Hv of HL161B
caactgttgctccaggaatccggtcctggtcttgtaaagccatctgagactctctcccttacctgtaccgttagcggaggaagtctttcctcaagcttctcctactgggtgtggatcagacagcctcccggaaaagggttggagtggattggcacaatatactactccggcaacacttactataaccccagcctgaagagcaggctgactatctctgtcgacaccagtaaaaatcacttttctctgaatctgtcttcagtgaccgcagccgacaccgccgtgtattattgcgctcggcgcgccgggattctgacaggctatctggattcatggggccaggggacattggttacagtgtctagt

SEQ ID NO: 4 - protein, 121 aa, Artificial Sequence
  Hv of HL161B
QLLLQESGPGLVKPSETLSLTCTVSGGSLSSSFSYWVWIRQPPGKGLEWIGTIYYSGNTYYNPSLKSRLTISVDTSKNHFSLNLSSVTAADTAVYYCARRAGILTGYLDSWGQGTLVTVSS

SEQ ID NO: 5 - DNA, 363 bp, Artificial Sequence
  Hv of HL161BK
cagctgctgctgcaagaatccggccctggcctggtgaaaccctccgagacactgtccctgacctgcaccgtgtccggcggctccctgtcctccagcttctcctactgggtctggatccggcagccccctggcaagggcctggaatggatcggcaccatctactactccggcaacacctactacaaccccagcctgaagtcccggctgaccatctccgtggacacctccaagaaccacttcagcctgaagctgtcctccgtgaccgccgctgacaccgccgtgtactactgtgccagaagggccggcatcctgaccggctacctggactcttggggccagggcaccctggtgacagtgtcctcc

SEQ ID NO: 6 - protein, 121 aa, Artificial Sequence
  Hv of HL161BK
QLLLQESGPGLVKPSETLSLTCTVSGGSLSSSFSYWVWIRQPPGKGLEWIGTIYYSGNTYYNPSLKSRLTISVDTSKNHFSLKLSSVTAADTAVYYCARRAGILTGYLDSWGQGTLVTVSS

SEQ ID NO: 7 - DNA, 354 bp, Artificial Sequence
  Hv of HL161C
caggtgcagctcgtgcagtccggcgcagaggtcaaaaagcctggtgcatctgtgaaagtgagttgcaaggctagcggctacacctttaccggatgttatatgcattgggtacgccaagcccccggacaaggcttggaatggatggggcgtatcaacccaaactctggcgggactaattacgcccagaagtttcagggaagggtgactatgacaagggacacatccatatccaccgcttatatggacctgtctcgactgcggtctgatgatacagccgtttattactgcgccagagactacagcggatggagcttcgattattgggggcagggtactttggtcacagtttcaagt

SEQ ID NO: 8 - protein, 118 aa, Artificial Sequence
  Hv of HL161C
QVQLVQSGAEVKKPGASVKVSCKASGYTFTGCYMHWVRQAPGQGLEWMGRINPNSGGTNYAQKFQGRVTMTRDTSISTAYMDLSRLRSDDTAVYYCARDYSGWSFDYWGQGTLVTVSS

SEQ ID NO: 9 - DNA, 369 bp, Artificial Sequence
  Hv of HL161D
cagctgcagttgcaggagtcaggccccggtttggttaagccttctgaaaccctttctctcacatgcacagtatccggtggctccatctccagttcaagttactactggggatggatccggcaacccccaggaaaagggctggagtggattggcaatatatattactctgggtccacctattacaacccttccctgatgagtagagtgaccatcagcgtggacacaagcaaaaaccaattcagcctgaagctttctagcgtgaccgctgccgacacagctgtctattactgtgcccgccagcttagttataactggaatgataggctgtttgattactggggccaggggactctcgttacagtcagcagc

SEQ ID NO: 10 - protein, 123 aa, Artificial Sequence
  Hv of HL161D
QLQLQESGPGLVKPSETLSLTCTVSGGSISSSSYYWGWIRQPPGKGLEWIGNIYYSGSTYYNPSLMSRVTISVDTSKNQFSLKLSSVTAADTAVYYCARQLSYNWNDRLFDYWGQGTLVTVSS

SEQ ID NO: 11 - DNA, 357 bp, Artificial Sequence
  Lv of HL161A
tcttacgtgctgacccagcccccctccgtgtctgtggctcctggccagaccgccagaatcacctgtggcggcaacaacatcggctccacctccgtgcactggtatcagcagaagcccggccaggcccccgtgctggtggtgcacgacgactccgaccggccttctggcatccctgagcggttctccggctccaactccggcaacaccgccaccctgaccatctccagagtggaagccggcgacgaggccgactactactgccaagtgcgagactcctcctccgaccacgtgatcttcggcggaggcaccaagctgaccgtgctgggccagcctaaggccgctccctccgtgaccctg

SEQ ID NO: 12 - protein, 119 aa, Artificial Sequence
  Lv of HL161A
SYVLTQPPSVSVAPGQTARITCGGNNIGSTSVHWYQQKPGQAPVLVVHDDSDRPSGIPERFSGSNSGNTATLTISRVEAGDEADYYCQVRDSSSDHVIFGGGTKLTVLGQPKAAPSVTL

SEQ ID NO: 13 - DNA, 357 bp, Artificial Sequence
  Lv of HL161B
tcttacgtgctgacccagtccccctccgtgtccgtggctcctggccagaccgccagaatcacctgtggcggcaacaacatcggctccaagtccgtgcactggtatcagcagaagcccggccaggcccccgtgctggtggtgtacgacgactccgaccggccctctggcatccctgagcggttctccgcctccaactccggcaacaccgccaccctgaccatctccagagtggaagccggcgacgaggccgactactactgccaagtgtgggactcctcctccgaccacgtggtgttcggcggaggcaccaagctgaccgtgctgggccagcctaaggccgctccctccgtgaccctg

SEQ ID NO: 14 - protein, 119 aa, Artificial Sequence
  Lv of HL161B
SYVLTQSPSVSVAPGQTARITCGGNNIGSKSVHWYQQKPGQAPVLVVYDDSDRPSGIPERFSASNSGNTATLTISRVEAGDEADYYCQVWDSSSDHVVFGGGTKLTVLGQPKAAPSVTL

SEQ ID NO: 15 - DNA, 357 bp, Artificial Sequence; identical to SEQ ID NO: 13
  Lv of HL161BK

SEQ ID NO: 16 - protein, 119 aa, Artificial Sequence; identical to SEQ ID NO: 14
  Lv of HL161BK

SEQ ID NO: 17 - DNA, 351 bp, Artificial Sequence
  Lv of HL161C
gacatccagatgacccagtcaccatcatccctttccgcatctgtcggagatagagtgactatcacctgcagggcttctcaaggtatttccaactacctcgcctggttccagcaaaagccaggtaaagccccaaagagcttgatctacgccgcttctagtctgcagagtggagttcctagtaagttctccggctctggcagtggcacagattttaccttgaccatttccagcctgcagtctgaggatttcgctacctactattgtcagcagtatgacagctatccccccacatttggggggggcactaaggtggagataaaacggacagtggctgccccttctgtctttatt

SEQ ID NO: 18 - protein, 117 aa, Artificial Sequence
  Lv of HL161C
DIQMTQSPSSLSASVGDRVTITCRASQGISNYLAWFQQKPGKAPKSLIYAASSLQSGVPSKFSGSGSGTDFTLTISSLQSEDFATYYCQQYDSYPPTFGGGTKVEIKRTVAAPSVFI

SEQ ID NO: 19 - DNA, 351 bp, Artificial Sequence
  Lv of HL161D
agctatgagctgacccagcctctgagcgtatctgtcgctctcggccagacagccagaattacctgtggcggcaataacataggatccaaaaatgttcactggtatcagcaaaaacctggccaagctcccgtgctcgtgatctaccgggactctaaccgacccagtggaatccccgaacgctttagcggttccaactctggaaatacagctactctgactatctccagggctcaggccggggatgaggccgattactactgccaggtgtgggactcaagcacagtggtcttcggcggaggtaccaagttgactgttcttgggcagccaaaggccgcaccttcagtgaccctg

SEQ ID NO: 20 - protein, 117 aa, Artificial Sequence
  Lv of HL161D
SYELTQPLSVSVALGQTARITCGGNNIGSKNVHWYQQKPGQAPVLVIYRDSNRPSGIPERFSGSNSGNTATLTISRAQAGDEADYYCQVWDSSTVVFGGGTKLTVLGQPKAAPSVTL

SEQ ID NO: 21 - protein, 5 aa, Artificial Sequence
  Hv CDR1 of HL161A
SCVMT

SEQ ID NO: 22 - protein, 17 aa, Artificial Sequence
  Hv CDR2 of HL161A
VISGSGGSTYYADSVKG

SEQ ID NO: 23 - protein, 12 aa, Artificial Sequence
  Hv CDR3 of HL161A
TPWWLRSPFFDY

SEQ ID NO: 24 - protein, 11 aa, Artificial Sequence
  Lv CDR1 of HL161A
GGNNIGSTSVH

SEQ ID NO: 25 - protein, 7 aa, Artificial Sequence
  Lv CDR2 of HL161A
DDSDRPS

SEQ ID NO: 26 - protein, 10 aa, Artificial Sequence
  Lv CDR3 of HL161A
VRDSSSDHVI

SEQ ID NO: 27 - protein, 5 aa, Artificial Sequence
  Hv CDR1 of HL161B or HL161BK
FSYWV

SEQ ID NO: 28 - protein, 16 aa, Artificial Sequence
  Hv CDR2 of HL161B or HL161BK
TIYYSGNTYYNPSLKS

SEQ ID NO: 29 - protein, 11 aa, Artificial Sequence
  Hv CDR3 of HL161B or HL161BK
RAGILTGYLDS

SEQ ID NO: 30 - protein, 11 aa, Artificial Sequence
  Lv CDR1 of HL161B or HL161BK
GGNNIGSKSVH

SEQ ID NO: 31 - protein, 7 aa, Artificial Sequence
  Lv CDR2 of HL161B or HL161BK
DDSDRPS

SEQ ID NO: 32 - protein, 11 aa, Artificial Sequence
  Lv CDR3 of HL161B or HL161BK
QVWDSSSDHVV

SEQ ID NO: 33 - protein, 5 aa, Artificial Sequence
  Hv CDR1 of HL161C
GCYMH

SEQ ID NO: 34 - protein, 17 aa, Artificial Sequence
  Hv CDR2 of HL161C
RINPNSGGTNYAQKFQG

SEQ ID NO: 35 - protein, 9 aa, Artificial Sequence
  Hv CDR3 of HL161C
DYSGWSFDY

SEQ ID NO: 36 - protein, 11 aa, Artificial Sequence
  Lv CDR1 of HL161C
RASQGISNYLA

SEQ ID NO: 37 - protein, 7 aa, Artificial Sequence
  Lv CDR2 of HL161C
AASSLQS

SEQ ID NO: 38 - protein, 10 aa, Artificial Sequence
  Lv CDR3 of HL161C
QQYDSYPPTF

SEQ ID NO: 39 - protein, 5 aa, Artificial Sequence
  Hv CDR1 of HL161D
SYYWG

SEQ ID NO: 40 - protein, 16 aa, Artificial Sequence
  Hv CDR2 of HL161D
NIYYSGSTYYNPSLMS

SEQ ID NO: 41 - protein, 13 aa, Artificial Sequence
  Hv CDR3 of HL161D
QLSYNWNDRLFDY

SEQ ID NO: 42 - protein, 11 aa, Artificial Sequence
  Lv CDR1 of HL161D
GGNNIGSKNVH

SEQ ID NO: 43 - protein, 7 aa, Artificial Sequence
  Lv CDR2 of HL161D
RDSNRPS

SEQ ID NO: 44 - protein, 9 aa, Artificial Sequence
  Lv CDR3 of HL161D
QVWDSSTVV